European Patent Application EP 4 606 888 A1, published August 27, 2025. Title: A novel method for preparing neural stem cells/neural progenitor cells. Applicant: K Pharma, Inc. Application WO PCT/JP2023/ 37824, filed October 19, 2023. The sequence listing filed with the application follows.

SEQUENCE LISTING (22 sequences)

SEQ ID NO: 1 - DNA, 24 bp, synthetic construct
  misc_feature 1..24: note = Forward primer for PAX6 gene
  source 1..24: mol_type = other DNA
accacaccggtttcctccttcaca

SEQ ID NO: 2 - DNA, 22 bp, synthetic construct
  misc_feature 1..22: note = Reverse primer for PAX6 gene
  source 1..22: mol_type = other DNA
ttgccatggtgaagctgggcat

SEQ ID NO: 3 - DNA, 20 bp, synthetic construct
  misc_feature 1..20: note = Forward primer for SOX1 gene
  source 1..20: mol_type = other DNA
gatcagcaagcgcctggggg

SEQ ID NO: 4 - DNA, 21 bp, synthetic construct
  misc_feature 1..21: note = Reverse primer for SOX1 gene
  source 1..21: mol_type = other DNA
agcagcgtcttggtcttgcgg

SEQ ID NO: 5 - DNA, 24 bp, synthetic construct
  misc_feature 1..24: note = Forward primer for NESTIN gene
  source 1..24: mol_type = other DNA
ttccctcagctttcaggaccccaa

SEQ ID NO: 6 - DNA, 22 bp, synthetic construct
  misc_feature 1..22: note = Reverse primer for NESTIN gene
  source 1..22: mol_type = other DNA
aaggctggcacaggtgtctcaa

SEQ ID NO: 7 - DNA, 22 bp, synthetic construct
  misc_feature 1..22: note = Forward primer for OCT4 gene
  source 1..22: mol_type = other DNA
ttgggctcgagaaggatgtggt

SEQ ID NO: 8 - DNA, 22 bp, synthetic construct
  misc_feature 1..22: note = Reverse primer for OCT4 gene
  source 1..22: mol_type = other DNA
tgcatagtcgctgcttgatcgc

SEQ ID NO: 9 - DNA, 23 bp, synthetic construct
  misc_feature 1..23: note = Forward primer for SOX17 gene
  source 1..23: mol_type = other DNA
acgctttcatggtgtgggctaag

SEQ ID NO: 10 - DNA, 21 bp, synthetic construct
  misc_feature 1..21: note = Reverse primer for SOX17 gene
  source 1..21: mol_type = other DNA
gtcagcgccttccacgacttg

SEQ ID NO: 11 - DNA, 23 bp, synthetic construct
  misc_feature 1..23: note = Forward primer for T gene
  source 1..23: mol_type = other DNA
ccttcagcaaagtcaagctcacc

SEQ ID NO: 12 - DNA, 22 bp, synthetic construct
  misc_feature 1..22: note = Reverse primer for T gene
  source 1..22: mol_type = other DNA
tgaactgggtctcagggaagca

SEQ ID NO: 13 - DNA, 25 bp, synthetic construct
  misc_feature 1..25: note = Forward primer for TUJ1 gene
  source 1..25: mol_type = other DNA
atttcatctttggtcagagtggggc

SEQ ID NO: 14 - DNA, 22 bp, synthetic construct
  misc_feature 1..22: note = Reverse primer for TUJ1 gene
  source 1..22: mol_type = other DNA
tgcaggcagtcgcagttttcac

SEQ ID NO: 15 - DNA, 19 bp, synthetic construct
  misc_feature 1..19: note = Forward primer for MAP2 gene
  source 1..19: mol_type = other DNA
ggatcaacggagagctgac

SEQ ID NO: 16 - DNA, 20 bp, synthetic construct
  misc_feature 1..20: note = Seq16_MAP2_R
  source 1..20: mol_type = other DNA
tcaggactgctacagcctca

SEQ ID NO: 17 - DNA, 18 bp, synthetic construct
  misc_feature 1..18: note = Forward primer for OLIG2 gene
  source 1..18: mol_type = other DNA
ggcgcgcaactacatcct

SEQ ID NO: 18 - DNA, 19 bp, synthetic construct
  misc_feature 1..19: note = Reverse primer for OLIG2 gene
  source 1..19: mol_type = other DNA
cgctcaccagtcgcttcat

SEQ ID NO: 19 - DNA, 21 bp, synthetic construct
  misc_feature 1..21: note = Forward primer for NG2 gene
  source 1..21: mol_type = other DNA
ttgtcctgatggctaatgcct

SEQ ID NO: 20 - DNA, 19 bp, synthetic construct
  misc_feature 1..19: note = Reverse primer for NG2 gene
  source 1..19: mol_type = other DNA
tgggctgctcgatggtgta

SEQ ID NO: 21 - DNA, 19 bp, synthetic construct
  misc_feature 1..19: note = Forward primer for CD44 gene
  source 1..19: mol_type = other DNA
tggcacccgctatgtcgag

SEQ ID NO: 22 - DNA, 19 bp, synthetic construct
  misc_feature 1..19: note = Reverse primer for CD44 gene
  source 1..19: mol_type = other DNA
gtagcagggattctgtctg